European Patent Application EP 4 119 582 A1, published January 18, 2023. Title: COMBINATION THERAPY INVOLVING ANTIBODIES AGAINST CLAUDIN 18.2 FOR TREATMENT OF CANCER. Applicant: Astellas Pharma Inc. et al. The sequence listing filed with the application follows.

SEQUENCE LISTING (50 sequences)

SEQ ID NO: 1 - protein, 261 aa, Homo sapiens
MAVTACQGLGFVVSLIGIAGIIAATCMDQWSTQDLYNNPVTAVFNYQGLWRSCVRESSGFTECRGYFTLLGLPAMLQAVRALMIVGIVLGAIGLLVSIFALKCIRIGSMEDSAKANMTLTSGIMFIVSGLCAIAGVSVFANMLVTNFWMSTANMYTGMGGMVQTVQTRYTFGAALFVGWVAGGLTLIGGVMMCIACRGLAPEETNYKAVSYHASGHSVAYKPGGFKASTGFGSNTKNKKIYDGGARTEDEVQSYPSKHDYV

SEQ ID NO: 2 - protein, 261 aa, Homo sapiens
MSTTTCQVVAFLLSILGLAGCIAATGMDMWSTQDLYDNPVTSVFQYEGLWRSCVRQSSGFTECRPYFTILGLPAMLQAVRALMIVGIVLGAIGLLVSIFALKCIRIGSMEDSAKANMTLTSGIMFIVSGLCAIAGVSVFANMLVTNFWMSTANMYTGMGGMVQTVQTRYTFGAALFVGWVAGGLTLIGGVMMCIACRGLAPEETNYKAVSYHASGHSVAYKPGGFKASTGFGSNTKNKKIYDGGARTEDEVQSYPSKHDYV

SEQ ID NO: 3 - protein, 10 aa, Homo sapiens
DQWSTQDLYN

SEQ ID NO: 4 - protein, 11 aa, Homo sapiens
NNPVTAVFNYQ

SEQ ID NO: 5 - protein, 14 aa, Homo sapiens
STQDLYNNPVTAVF

SEQ ID NO: 6 - protein, 13 aa, Homo sapiens
TNFWMSTANMYTG

SEQ ID NO: 7 - protein, 13 aa, Homo sapiens
DSAKANMTLTSGI

SEQ ID NO: 8 - protein, 55 aa, Homo sapiens
MDQWSTQDLYNNPVTAVFNYQGLWRSCVRESSGFTECRGYFTLLGLPAMLQAVRA

SEQ ID NO: 9 - protein, 24 aa, Homo sapiens
FALKCIRIGSMEDSAKANMTLTSG

SEQ ID NO: 10 - protein, 40 aa, Homo sapiens
ANMLVTNFWMSTANMYTGMGGMVQTVQTRYTFGAALFVGW

SEQ ID NO: 11 - protein, 153 aa, Homo sapiens
MDQWSTQDLYNNPVTAVFNYQGLWRSCVRESSGFTECRGYFTLLGLPAMLQAVRALMIVGIVLGAIGLLVSIFALKCIRIGSMEDSAKANMTLTSGIMFIVSGLCAIAGVSVFANMLVTNFWMSTANMYTGMGGMVQTVQTRYTFGAALFVGW

SEQ ID NO: 12 - protein, 107 aa, Artificial [sequence omitted]

SEQ ID NO: 13 - protein, 326 aa, Artificial
  Description of artificial sequence: Translation of PCR product
GPSVFPLAPSSKSTSGGTAALGCLVKDYFPEPVTVSWNSGALTSGVHTFPAVLQSSGLYSLSSVVTVPSSSLGTQTYICNVNHKPSNTKVDKKVEPKSCDKTHTCPPCPAPELLGGPSVFLFPPKPKDTLMISRTPEVTCVVVDVSHEDPEVKFNWYVDGVEVHNAKTKPREEQYNSTYRVVSVLTVLHQDWLNGKEYKCKVSNKALPAPIEKTISKAKGQPREPQVYTLPPSRDELTKNQVSLTCLVKGFYPSDIAVEWESNGQPENNYKTTPPVLDSDGSFFLYSKLTVDKSRWQQGNVFSCSVMHEALHNHYTQKSLSLSPGK

SEQ ID NO: 14 - protein, 466 aa, Artificial
  Description of artificial sequence: chimeric monoclonal antibody
MEWTWVFLFLLSVTAGVHSQVQLQQSGAELMKPGASVKISCKATGYTFSSYWIEWVKQRPGHGLEWIGEILPGSGSTNYNEKFKGKATFTADTSSNTAYMQLSSLTSEDSAVYYCARYDYPWFAYWGQGTLVTVSAASTKGPSVFPLAPSSKSTSGGTAALGCLVKDYFPEPVTVSWNSGALTSGVHTFPAVLQSSGLYSLSSVVTVPSSSLGTQTYICNVNHKPSNTKVDKKVEPKSCDKTHTCPPCPAPELLGGPSVFLFPPKPKDTLMISRTPEVTCVVVDVSHEDPEVKFNWYVDGVEVHNAKTKPREEQYNSTYRVVSVLTVLHQDWLNGKEYKCKVSNKALPAPIEKTISKAKGQPREPQVYTLPPSRDELTKNQVSLTCLVKGFYPSDIAVEWESNGQPENNYKTTPPVLDSDGSFFLYSKLTVDKSRWQQGNVFSCSVMHEALHNHYTQKSLSLSPGK

SEQ ID NO: 15 - protein, 467 aa, Artificial
  Description of artificial sequence: chimeric monoclonal antibody
MDWLWNLLFLMAAAQSIQAQIQLVQSGPELKKPGETVKISCKASGYTFTNYGMNWVKQAPGKGLKWMGWINTNTGEPTYAEEFKGRFAFSLETSASTAYLQINNLKNEDTATYFCARLGFGNAMDYWGQGTSVTVSSASTKGPSVFPLAPSSKSTSGGTAALGCLVKDYFPEPVTVSWNSGALTSGVHTFPAVLQSSGLYSLSSVVTVPSSSLGTQTYICNVNHKPSNTKVDKKVEPKSCDKTHTCPPCPAPELLGGPSVFLFPPKPKDTLMISRTPEVTCVVVDVSHEDPEVKFNWYVDGVEVHNAKTKPREEQYNSTYRVVSVLTVLHQDWLNGKEYKCKVSNKALPAPIEKTISKAKGQPREPQVYTLPPSRDELTKNQVSLTCLVKGFYPSDIAVEWESNGQPENNYKTTPPVLDSDGSFFLYSKLTVDKSRWQQGNVFSCSVMHEALHNHYTQKSLSLSPGK

SEQ ID NO: 16 - protein, 465 aa, Artificial
  Description of artificial sequence: chimeric monoclonal antibody
MEWIWIFLFILSGTAGVHSQVQLQQSGAELARPGASVKLSCKASGYTFTDYYINWVKQRTGQGLEWIGEIYPGSGNTYYNEKFKGKATLTADKSSSTAYMQLSSLTSEDSAVYFCARSYGAFDYWGQGTTLTVSSASTKGPSVFPLAPSSKSTSGGTAALGCLVKDYFPEPVTVSWNSGALTSGVHTFPAVLQSSGLYSLSSVVTVPSSSLGTQTYICNVNHKPSNTKVDKKVEPKSCDKTHTCPPCPAPELLGGPSVFLFPPKPKDTLMISRTPEVTCVVVDVSHEDPEVKFNWYVDGVEVHNAKTKPREEQYNSTYRVVSVLTVLHQDWLNGKEYKCKVSNKALPAPIEKTISKAKGQPREPQVYTLPPSRDELTKNQVSLTCLVKGFYPSDIAVEWESNGQPENNYKTTPPVLDSDGSFFLYSKLTVDKSRWQQGNVFSCSVMHEALHNHYTQKSLSLSPGK

SEQ ID NO: 17 - protein, 467 aa, Artificial
  Description of artificial sequence: chimeric monoclonal antibody
MGWSCIILFLVATATGVHSQVQLQQPGAELVRPGASVKLSCKASGYTFTSYWINWVKQRPGQGLEWIGNIYPSDSYTNYNQKFKDKATLTVDKSSSTAYMQLSSPTSEDSAVYYCTRSWRGNSFDYWGQGTTLTVSSASTKGPSVFPLAPSSKSTSGGTAALGCLVKDYFPEPVTVSWNSGALTSGVHTFPAVLQSSGLYSLSSVVTVPSSSLGTQTYICNVNHKPSNTKVDKKVEPKSCDKTHTCPPCPAPELLGGPSVFLFPPKPKDTLMISRTPEVTCVVVDVSHEDPEVKFNWYVDGVEVHNAKTKPREEQYNSTYRVVSVLTVLHQDWLNGKEYKCKVSNKALPAPIEKTISKAKGQPREPQVYTLPPSRDELTKNQVSLTCLVKGFYPSDIAVEWESNGQPENNYKTTPPVLDSDGSFFLYSKLTVDKSRWQQGNVFSCSVMHEALHNHYTQKSLSLSPGK

SEQ ID NO: 18 - protein, 466 aa, Artificial
  Description of artificial sequence: chimeric monoclonal antibody
MEWRIFLFILSGTAGVHSQVQLQQSGPELVKPGASVKMSCKASGYTFTDYVISWVKQRTGQGLEWIGEIYPGSGSTYYNEKFKGKATLTADKSSNTAYMQLSSLTSEDSAVYFCARGVLLRAMDYWGQGTSVTVSSASTKGPSVFPLAPSSKSTSGGTAALGCLVKDYFPEPVTVSWNSGALTSGVHTFPAVLQSSGLYSLSSVVTVPSSSLGTQTYICNVNHKPSNTKVDKKVEPKSCDKTHTCPPCPAPELLGGPSVFLFPPKPKDTLMISRTPEVTCVVVDVSHEDPEVKFNWYVDGVEVHNAKTKPREEQYNSTYRVVSVLTVLHQDWLNGKEYKCKVSNKALPAPIEKTISKAKGQPREPQVYTLPPSRDELTKNQVSLTCLVKGFYPSDIAVEWESNGQPENNYKTTPPVLDSDGSFFLYSKLTVDKSRWQQGNVFSCSVMHEALHNHYTQKSLSLSPGK

SEQ ID NO: 19 - protein, 469 aa, Artificial [sequence omitted]

SEQ ID NO: 20 - protein, 240 aa, Artificial
  Description of artificial sequence: chimeric monoclonal antibody
MESQTQVLMSLLFWVSGTCGDIVMTQSPSSLTVTAGEKVTMSCKSSQSLLNSGNQKNYLTWYQQKPGQPPKLLIYWASTRESGVPDRFTGSGSGTDFTLTISSVQAEDLAVYYCQNDYSYPLTFGAGTKLELKRTVAAPSVFIFPPSDEQLKSGTASVVCLLNNFYPREAKVQWKVDNALQSGNSQESVTEQDSKDSTYSLSSTLTLSKADYEKHKVYACEVTHQGLSSPVTKSFNRGEC

SEQ ID NO: 21 - protein, 235 aa, Artificial
  Description of artificial sequence: chimeric monoclonal antibody
MHFQVQIFSFLLISASVIMSRGQIVLTQSPAIMSASPGEKVTITCSASSSVSYMHWFQQKPGTSPKLWIYSTSNLASGVPARFSGSGSGTSYSLTISRMEAEDAATYYCQQRSSYPPTFGGGTKLEIKRTVAAPSVFIFPPSDEQLKSGTASVVCLLNNFYPREAKVQWKVDNALQSGNSQESVTEQDSKDSTYSLSSTLTLSKADYEKHKVYACEVTHQGLSSPVTKSFNRGEC

SEQ ID NO: 22 - protein, 234 aa, Artificial
  Description of artificial sequence: chimeric monoclonal antibody
MEFQTQVFVFVLLWLSGVDGDIVMTQSQKFMSTSVGDRVSITCKASQNVRTAVAWYQQKPGQSPKALIYLASNRHTGVPDRFTGSGSGTDFTLTISNVQSEDLADYFCLQHWNYPLTFGGGTKLEIKRTVAAPSVFIFPPSDEQLKSGTASVVCLLNNFYPREAKVQWKVDNALQSGNSQESVTEQDSKDSTYSLSSTLTLSKADYEKHKVYACEVTHQGLSSPVTKSFNRGEC

SEQ ID NO: 23 - protein, 240 aa, Artificial
  Description of artificial sequence: chimeric monoclonal antibody
MDSQAQVLMLLLLWVSGTCGDIVMSQSPSSLAVSVGEKVTMSCKSSQSLLYSSNQKNYLAWYQQKPGQSPKLLIYWASTRESGVPDRFTGSGSGTDFTLTISSVKAEDLAVYYCQQYYSYPLTFGAGTKLELKRTVAAPSVFIFPPSDEQLKSGTASVVCLLNNFYPREAKVQWKVDNALQSGNSQESVTEQDSKDSTYSLSSTLTLSKADYEKHKVYACEVTHQGLSSPVTKSFNRGEC

SEQ ID NO: 24 - protein, 240 aa, Artificial
  Description of artificial sequence: chimeric monoclonal antibody
MESQTQVLMSLLFWVSGTCGDIVMTQSPSSLTVTAGEKVTMSCKSSQSLLNSGNQKNYLTWYQQKPGQPPKLLIYWASTRESGVPDRFTGSGSGTDFTLTISSVQAEDLAVYYCQNDYSYPFTFGSGTKLEIKRTVAAPSVFIFPPSDEQLKSGTASVVCLLNNFYPREAKVQWKVDNALQSGNSQESVTEQDSKDSTYSLSSTLTLSKADYEKHKVYACEVTHQGLSSPVTKSFNRGEC

SEQ ID NO: 25 - protein, 239 aa, Artificial
  Description of artificial sequence: chimeric monoclonal antibody
MDSQAQVLILLLLWVSGTCGDIVMSQSPSSLAVSAGEKVTMSCKSSQSLLNSRTRKNYLAWYQQKPGQSPKLLIYWASTRESGVPDRFTGSGSGTDFTLTISSVQAEDLAVYYCKQSYNLYTFGGGTKLEIKRTVAAPSVFIFPPSDEQLKSGTASVVCLLNNFYPREAKVQWKVDNALQSGNSQESVTEQDSKDSTYSLSSTLTLSKADYEKHKVYACEVTHQGLSSPVTKSFNRGEC

SEQ ID NO: 26 - protein, 240 aa, Artificial
  Description of artificial sequence: chimeric monoclonal antibody
MDSQAQVLMLLLLWVSGTCGDIVMSQSPSSLAVSVGEKVTMSCKSSQSLLYSSNQKNYLAWYQQKPGQSPKLLIYWASTRESGVPDRFTGSGSATDFTLTISSVQAEDLADYHCGQGYSYPYTFGGGTKLEIKRTVAAPSVFIFPPSDEQLKSGTASVVCLLNNFYPREAKVQWKVDNALQSGNSQESVTEQDSKDSTYSLSSTLTLSKADYEKHKVYACEVTHQGLSSPVTKSFNRGEC

SEQ ID NO: 27 - protein, 240 aa, Artificial; identical to SEQ ID NO: 23
  Description of artificial sequence: chimeric monoclonal antibody

SEQ ID NO: 28 - protein, 234 aa, Artificial
  Description of artificial sequence: chimeric monoclonal antibody
MESQTLVFISILLWLYGADGNIVMTQSPKSMSMSVGERVTLTCKASENVVTYVSWYQQKPEQSPKLLIYGASNRYTGVPDRFTGSGSATDFTLTISSVKAEDLAVYYCQQYYSYPLTFGAGTKLELKRTVAAPSVFIFPPSDEQLKSGTASVVCLLNNFYPREAKVQWKVDNALQSGNSQESVTEQDSKDSTYSLSSTLTLSKADYEKHKVYACEVTHQGLSSPVTKSFNRGEC

SEQ ID NO: 29 - protein, 117 aa, Artificial
  Description of artificial sequence: Translation of PCR product
QVQLQQSGAELMKPGASVKISCKATGYTFSSYWIEWVKQRPGHGLEWIGEILPGSGSTNYNEKFKGKATFTADTSSNTAYMQLSSLTSEDSAVYYCARYDYPWFAYWGQGTLVTVSA

SEQ ID NO: 30 - protein, 118 aa, Artificial
  Description of artificial sequence: Translation of PCR product
QIQLVQSGPELKKPGETVKISCKASGYTFTNYGMNWVKQAPGKGLKWMGWINTNTGEPTYAEEFKGRFAFSLETSASTAYLQINNLKNEDTATYFCARLGFGNAMDYWGQGTSVTVSS

SEQ ID NO: 31 - protein, 116 aa, Artificial
  Description of artificial sequence: Translation of PCR product
QVQLQQSGAELARPGASVKLSCKASGYTFTDYYINWVKQRTGQGLEWIGEIYPGSGNTYYNEKFKGKATLTADKSSSTAYMQLSSLTSEDSAVYFCARSYGAFDYWGQGTTLTVSS

SEQ ID NO: 32 - protein, 118 aa, Artificial
  Description of artificial sequence: Translation of PCR product
QVQLQQPGAELVRPGASVKLSCKASGYTFTSYWINWVKQRPGQGLEWIGNIYPSDSYTNYNQKFKDKATLTVDKSSSTAYMQLSSPTSEDSAVYYCTRSWRGNSFDYWGQGTTLTVSS

SEQ ID NO: 33 - protein, 118 aa, Artificial
  Description of artificial sequence: Translation of PCR product
QVQLQQSGPELVKPGASVKMSCKASGYTFTDYVISWVKQRTGQGLEWIGEIYPGSGSTYYNEKFKGKATLTADKSSNTAYMQLSSLTSEDSAVYFCARGVLLRAMDYWGQGTSVTVSS

SEQ ID NO: 34 - protein, 120 aa, Artificial
  Description of artificial sequence: Translation of PCR product
QVHLQQSGSELRSPGSSVKLSCKDFDSEVFPFAYMSWIRQKPGHGFEWIGDILPSIGRTIYGEKFEDKATLDADTVSNTAYLELNSLTSEDSAIYYCARGEGYGAWFAYWGQGTLVTVSA

SEQ ID NO: 35 - protein, 113 aa, Artificial
  Description of artificial sequence: Translation of PCR product
DIVMTQSPSSLTVTAGEKVTMSCKSSQSLLNSGNQKNYLTWYQQKPGQPPKLLIYWASTRESGVPDRFTGSGSGTDFTLTISSVQAEDLAVYYCQNDYSYPLTFGAGTKLELK

SEQ ID NO: 36 - protein, 106 aa, Artificial
  Description of artificial sequence: Translation of PCR product
QIVLTQSPAIMSASPGEKVTITCSASSSVSYMHWFQQKPGTSPKLWIYSTSNLASGVPARFSGSGSGTSYSLTISRMEAEDAATYYCQQRSSYPPTFGGGTKLEIK

SEQ ID NO: 37 - protein, 107 aa, Artificial
  Description of artificial sequence: Translation of PCR product
DIVMTQSQKFMSTSVGDRVSITCKASQNVRTAVAWYQQKPGQSPKALIYLASNRHTGVPDRFTGSGSGTDFTLTISNVQSEDLADYFCLQHWNYPLTFGGGTKLEIK

SEQ ID NO: 38 - protein, 113 aa, Artificial
  Description of artificial sequence: Translation of PCR product
DIVMSQSPSSLAVSVGEKVTMSCKSSQSLLYSSNQKNYLAWYQQKPGQSPKLLIYWASTRESGVPDRFTGSGSGTDFTLTISSVKAEDLAVYYCQQYYSYPLTFGAGTKLELK

SEQ ID NO: 39 - protein, 113 aa, Artificial
  Description of artificial sequence: Translation of PCR product
DIVMTQSPSSLTVTAGEKVTMSCKSSQSLLNSGNQKNYLTWYQQKPGQPPKLLIYWASTRESGVPDRFTGSGSGTDFTLTISSVQAEDLAVYYCQNDYSYPFTFGSGTKLEIK

SEQ ID NO: 40 - protein, 112 aa, Artificial
  Description of artificial sequence: Translation of PCR product
DIVMSQSPSSLAVSAGEKVTMSCKSSQSLLNSRTRKNYLAWYQQKPGQSPKLLIYWASTRESGVPDRFTGSGSGTDFTLTISSVQAEDLAVYYCKQSYNLYTFGGGTKLEIK

SEQ ID NO: 41 - protein, 113 aa, Artificial
  Description of artificial sequence: Translation of PCR product
DIVMSQSPSSLAVSVGEKVTMSCKSSQSLLYSSNQKNYLAWYQQKPGQSPKLLIYWASTRESGVPDRFTGSGSATDFTLTISSVQAEDLADYHCGQGYSYPYTFGGGTKLEIK

SEQ ID NO: 42 - protein, 113 aa, Artificial; identical to SEQ ID NO: 38
  Description of artificial sequence: Translation of PCR product

SEQ ID NO: 43 - protein, 107 aa, Artificial
  Description of artificial sequence: Translation of PCR product
NIVMTQSPKSMSMSVGERVTLTCKASENVVTYVSWYQQKPEQSPKLLIYGASNRYTGVPDRFTGSGSATDFTLTISSVKAEDLAVYYCQQYYSYPLTFGAGTKLELK

SEQ ID NO: 44 - protein, 15 aa, Artificial
  Epitope
MDQWSTQDLYNNPVT

SEQ ID NO: 45 - protein, 15 aa, Artificial
  Epitope
STQDLYNNPVTAVFN

SEQ ID NO: 46 - protein, 15 aa, Artificial
  Epitope
LYNNPVTAVFNYQGL

SEQ ID NO: 47 - protein, 15 aa, Artificial
  Epitope
PVTAVFNYQGLWRSC

SEQ ID NO: 48 - protein, 15 aa, Artificial
  Epitope
VFNYQGLWRSCVRES

SEQ ID NO: 49 - protein, 15 aa, Artificial
  Epitope
QGLWRSCVRESSGFT

SEQ ID NO: 50 - protein, 15 aa, Artificial
  Epitope
RSCVRESSGFTECRG